European Patent Application EP 4 362 028 A1, published May 1, 2024. Title: Mutant Aerolysin and uses thereof. Applicant: ECOLE POLYTECHNIQUE FEDERALE DE LAUSANNE (EPFL). Application EP. The sequence listing filed with the application follows.

SEQUENCE LISTING (19 sequences)

SEQ ID NO: 1 - protein, 470 aa, Aeromonas hydrophila
AEPVYPDQLRLFSLGQGVCGDKYRPVNREEAQSVKSNIVGMMGQWQISGLANGWVIMGPGYNGEIKPGTASNTWCYPTNPVTGEIPTLSALDIPDGDEVDVQWRLVHDSANFIKPTSYLAHYLGYAWVGGNHSQYVGEDMDVTRDGDGWVIRGNNDGGCDGYRCGDKTAIKVSNFAYNLDPDSFKHGDVTQSDRQLVKTVVGWAVNDSDTPQSGYDVTLRYDTATNWSKTNTYGLSEKVTTKNKFKWPLVGETELSIEIAANQSWASQNGGSTTTSLSQSVRPTVPARSKIPVKIELYKADISYPYEFKADVSYDLTLSGFLRWGGNAWYTHPDNRPNWNHTFVIGPYKDKASSIRYQWDKRYIPGEVKWWDWNWTIQQNGLSTMQNNLARVLRPVRAGITGDFSAESQFAGNIEIGAPVPLAADSKVRRARSVDGAGQGLRLEIPLDAQELSGLGFNNVSLSVTPAANQ

SEQ ID NO: 2 - protein, 462 aa, Aeromonas hydrophila
AEPVYPDQLRLFSLGQEVCGDKYRPITREEAQSVKSNIVNMMGQWQISGLANGWVIMGPVYNGEIKPGSASNTWCYPVNPVTGEIPTLSALDIPDGDEVDVQWRLVHDSANFIKPTSYLAHYLGYAWVGGNHSQYVGEDMDVTRDGDGWVIRGNNDGGCEGYRCGEKTAIKVSNFAYNLDPDSFKHGDVTQSDRQLVKTVVGWAINDSYTPQSAYDVTLRYDTATNWSKTNTYGLSEKVTTKNKFKWPLVGETELSIEIAANQSWASQNGGSTTTSLSQSVRPTVPARSKIPVKIELYKADISYPYEFKADVSYDLTLSGFLRWGGNAWYTHPDNRPNWNHTFVIGPYKDKASSIRYQWDKRYIPGEVKWWDWNWTIQQNGLSTMQNNLARVLRPVRAGITGDFSAESQFAGNIEIGAPVPLAADGKAPRALSARRGEQGLRLAIPLECRKSSPGLASATSA

SEQ ID NO: 3 - protein, 464 aa, Aeromonas sobria
AEPVYPDQVKWAGLGTGVCASGYRPLTRDEAMSIKGNLVSRMGQWQITGLADRWVIMGPGYNGEIKQGTAGETWCYPNSPVSGEIPTLSDWNIPAGDEVDVQWRLVHDNDYFIKPVSYLAHYLGYAWVGGNHSPYVGEDMDVTRVGDGWLIKGNNDGGCSGYRCGEKSSIKVSNFSYTLEPDSFSHGQVTESGKQLVKTITANATNYTDLPQQVVVTLKYDKATNWSKTDTYSLSEKVTTKNKFQWPLVGETELAIEIAASQSWASQKGGSTTETVSVEARPTVPPHSSLPVRVALYKSNISYPYEFKAEVNYDLTMKGFLRWGGNAWYTHPDNRPTWEHTLLLGPFRGQGEQHPLPVDKRYIPGEVKWWDWNWTISEYGLSTMQNNLGRVLRPIRSAVTGDFYAESQFAGDIEIGQPQTRSAKAAQLRSASAEEVALTSVDLDSEALANEGFGNVSLTIVPVQ

SEQ ID NO: 4 - protein, 469 aa, Aeromonas hydrophila
AEPVYPDQLRLFSLGQEVCGDKYRPVNREEAQSVKSNIVGMMGQWQISGLANGWVIMGPGYNGEIKPGSASSTWCYPTNPATGEIPTLSALDIPDGDEVDVQWRLVHDSANFIKPTSYLAHYLGYAWVGGNHSQYVGEDMDVTRDGDGWVIRGNNDGGCDGYRCGDKTSIKVSNFAYNLDPDSFKHGDVTQSDRQLVKTVVGWAINDSDTPQSGYDVTLRYDTATNWSKTNTYGLSEKVTTKNKFKWPLVGETELSIEIAANQSWASQNGGSPTTSLSQSVRPTVPAHSKIPVKIELYKADISYPYEFKADVSYDLTLSGFLRWGGNAWYTHPDNRPNWNHTFVIGPYKDKASSIRYQWDKRYIPGEVKWWDWNWTIQQNGLPTMQNNLAKVLRPVRAGITGDFSAESQFAGNIEIGAPVPVAAASHSSRARNLSAGQGLRLEIPLDAQELSGLGFNNVSLSVTPAANQ

SEQ ID NO: 5 - protein, 471 aa, Aeromonas enteropelogenes
NAAEPIYPDQLRLFSLGEDVCGTDYRPINREEAQSVRNNIVAMMGQWQISGLANNWVILGPGYNGEIKPGKASTTWCYPTRPATAEIPVLPAFNIPDGDAVDVQWRMVHDSANFIKPVSYLAHYLGYAWVGGDHSQFVGDDMDVIQEGDDWVLRGNDGGKCDGYRCNEKSSIRVSNFAYTLDPGSFSHGDVTQSERTLVHTVVGWATNISDTPQSGYDVTLNYTTMSNWSKTNTYGLSEKVSTKNKFKWPLVGETEVSIEIAANQSWASQNGGAVTTALSQSVRPVVPARSRVPVKIELYKANISYPYEFKADMSYDLTFNGFLRWGGNAWHTHPEDRPTLSHTFAIGPFKDKASSIRYQWDKRYLPGEMKWWDWNWAIQQNGLATMQDSLARVLRPVRASITGDFRAESQFAGNIEIGTPVPLGSDSKVRRTRSVDGANTGLKLDIPLDAQELAELGFENVTLSVTPARN

SEQ ID NO: 6 - protein, 465 aa, Aeromonas salmonicida
WHEPVYPDQVKWAGLGTGVCASGYRPLTRDEAMSIKGNLVSRMGQWQITGLADRWVIMGPGYNGEIKQGTAGETWCYPNSPVSGEIPTLSDWNIPAGDEVDVQWRLVHDNDYFIKPVSYLAHYLGYAWVGGNHSPYVGEDMDVTRVGDGWLIKGNNDGGCSGYRCGEKSSIKVSNFSYTLEPDSFSHGQVTESGKQLVKTITANATNYTDLPQQVVVTLKYDKATNWSKTDTYSLSEKVTTKNKFQWPLVGETELAIEIAASQSWASQKGGSTTETVSVEARPTVPPHSSLPVRVALYKSNISYPYEFKAEVNYDLTMKGFLRWGGNAWYTHPDNRPTWEHTFRLGPFRGQGEQHPLPVDKRYIPGEVKWWDWNWTISEYGLSTMQNNLGRVLRPIRSAVTGDFYAESQFAGDIEIGQPQTRSAKAAQLRSASAEEVALTSVDLDSEALANEGFGNVSLTIVPVQ

SEQ ID NO: 7 - protein, 469 aa, Aeromonas hydrophila
AEPVYPDQLRLFSLGQEVCGDKYRPVNREEAQSIKSNIVGMMGQWQISGLANGWVIMGPGYNGEIKPGSASSTWCYPTNPATGEIPTLSALDIPDGDEVDVQWRLVHDSANFIKPTSYLAHYLGYAWVGGNHSQYVGEDMDVTRDGDGWVIRGNNDGGCDGYRCGDKTSIKVSNFAYNLDPDSFKHGDVTQSDRQLVKTVVGWAINDSDTPQSGYDVTLRYDTATNWSKTNTYGLSEKVTTKNKFKWPLVGETELSIEIAANQSWASQNGGSTTTSLSQSVRPTVPAHSKIPVKIELYKADISYPYEFKADVSYDLTLSGFLRWGGNAWYTHPDNRPNWNHTFVIGPYKDKASSIRYQWDKRYIPGEVKWWDWNWTIQQNGLPTMQNNLAKVLRPVRAGITGDFSAESQFAGNIEIGAPVPVAAASHSSRARNLSAGQGLRLEIPLDAQELSGLGFNNVSLSVTPAANQ

SEQ ID NO: 8 - protein, 422 aa, Aeromonas hydrophila
AEPVYPDQLRLFSLGQGVCGDKYRPVNREEAQSVKSNIVGMMGQWQISGLANGWVIMGPGYNGEIKPGTASNTWCYPTNPVTGEIPTLSALDIPDGDEVDVQWRLVHDSANFIKPTSYLAHYLGYAWVGGNHSQYVGEDMDVTRDGDGWVIRGNNDGGCDGYRCGDKTAIKVSNFAYNLDPDSFKHGDVTQSDRQLVKTVVGWAVNDSDTPQSGYDVTLRYDTATNWSKTNTYGLSEKVTTKNKFKWPLVGETELSIEIAANQSWASQNGGSTTTSLSQSVRPTVPARSKIPVKIELYKADISYPYEFKADVSYDLTLSGFLRWGGNAWYTHPDNRPNWNHTFVIGPYKDKASSIRYQWDKRYIPGEVKWWDWNWTIQQNGLSTMQNNLARVLRPVRAGITGDFSAESQFAGNIEIGAPVPL

SEQ ID NO: 9 - DNA, 1392 bp, Aeromonas hydrophila
  source 1..1392: mol_type = genomic DNA
gcagagcccgtctatccagaccagcttcgcttgttttcattgggccaaggggtctgtggcgacaagtatcgccccgtcaatcgagaagaagcccaaagcgttaaaagcaatattgtcggcatgatggggcaatggcaaataagcgggctggccaacggctgggtcattatggggccgggttataacggtgaaataaaaccagggacagcgtccaatacctggtgttatccgaccaatcctgttaccggtgaaataccgacactgtctgccctggatattccagatggtgacgaagtcgatgtgcagtggcgactggtacatgacagtgcgaatttcatcaaaccaaccagctatctggcccattacctcggttatgcctgggtgggcggcaatcacagccaatatgtcggcgaagacatggatgtgacccgtgatggcgacggctgggtgatccgtggcaacaatgacggcggctgtgacggctatcgctgtggtgacaagacggccatcaaggtcagcaacttcgcctataacctggatcccgacagcttcaagcatggcgatgtcacccagtccgaccgccagctggtcaagactgtggtgggctgggcggtcaacgacagcgacaccccccaatccggctatgacgtcaccctgcgctacgacacagccaccaactggtccaagaccaacacctatggcctgagcgagaaggtgaccaccaagaacaagttcaagtggccactggtgggggaaacccaactctccatcgagattcgtgccaatcagtcctgggcgtcccagaacgggggctcgaccaccacctccctgtctcagtccgtgcgaccgactgtgccggcccgctccaagatcccggtgaagatagagctctacaaggccgacatctcctatccctatgagttcaaggccgatgtcagctatgacctgaccctgagcggcttcctgcgctggggcggcaacgcctggtatacccacccggacaaccgtccgaactggaaccacaccttcgtcataggtccgtacaaggacaaggcgagcagcattcgctaccagtgggacaagcgttacatcccgggtgaagtgaagtggtgggactggaactggaccatacagcagaacggtctgtctaccatgcagaacaacctggccagagtgctgcgcccggtgcgggcggggatcaccggtgatttcagtgccgagagccagtttgccggcaacatagagatcggtgctcccgtgccgctcgcggctgacagcaaggtgcgtcgtgctcgcagtgtggacggcgctggtcaaggcctgaggctggagatcccgctcgatcgcgaagagctctccgggcttggcttcaacaagtcagcctcagcgtga

SEQ ID NO: 10 - protein, 422 aa, Aeromonas hydrophila
AEPVYPDQLRLFSLGQEVCGDKYRPITREEAQSVKSNIVNMMGQWQISGLANGWVIMGPVYNGEIKPGSASNTWCYPVNPVTGEIPTLSALDIPDGDEVDVQWRLVHDSANFIKPTSYLAHYLGYAWVGGNHSQYVGEDMDVTRDGDGWVIRGNNDGGCEGYRCGEKTAIKVSNFAYNLDPDSFKHGDVTQSDRQLVKTVVGWAINDSYTPQSAYDVTLRYDTATNWSKTNTYGLSEKVTTKNKFKWPLVGETELSIEIAANQSWASQNGGSTTTSLSQSVRPTVPARSKIPVKIELYKADISYPYEFKADVSYDLTLSGFLRWGGNAWYTHPDNRPNWNHTFVIGPYKDKASSIRYQWDKRYIPGEVKWWDWNWTIQQNGLSTMQNNLARVLRPVRAGITGDFSAESQFAGNIEIGAPVPL

SEQ ID NO: 11 - protein, 419 aa, Aeromonas sobria
AEPVYPDQVKWAGLGTGVCASGYRPLTRDEAMSIKGNLVSRMGQWQITGLADRWVIMGPGYNGEIKQGTAGETWCYPNSPVSGEIPTLSDWNIPAGDEVDVQWRLVHDNDYFIKPVSYLAHYLGYAWVGGNHSPYVGEDMDVTRVGDGWLIKGNNDGGCSGYRCGEKSSIKVSNFSYTLEPDSFSHGQVTESGKQLVKTITANATNYTDLPQQVVVTLKYDKATNWSKTDTYSLSEKVTTKNKFQWPLVGETELAIEIAASQSWASQKGGSTTETVSVEARPTVPPHSSLPVRVALYKSNISYPYEFKAEVNYDLTMKGFLRWGGNAWYTHPDNRPTWEHTLLLGPFRGQGEQHPLPVDKRYIPGEVKWWDWNWTISEYGLSTMQNNLGRVLRPIRSAVTGDFYAESQFAGDIEIGQPQ

SEQ ID NO: 12 - protein, 422 aa, Aeromonas hydrophila
AEPVYPDQLRLFSLGQEVCGDKYRPVNREEAQSVKSNIVGMMGQWQISGLANGWVIMGPGYNGEIKPGSASSTWCYPTNPATGEIPTLSALDIPDGDEVDVQWRLVHDSANFIKPTSYLAHYLGYAWVGGNHSQYVGEDMDVTRDGDGWVIRGNNDGGCDGYRCGDKTSIKVSNFAYNLDPDSFKHGDVTQSDRQLVKTVVGWAINDSDTPQSGYDVTLRYDTATNWSKTNTYGLSEKVTTKNKFKWPLVGETELSIEIAANQSWASQNGGSPTTSLSQSVRPTVPAHSKIPVKIELYKADISYPYEFKADVSYDLTLSGFLRWGGNAWYTHPDNRPNWNHTFVIGPYKDKASSIRYQWDKRYIPGEVKWWDWNWTIQQNGLPTMQNNLAKVLRPVRAGITGDFSAESQFAGNIEIGAPVPV

SEQ ID NO: 13 - protein, 424 aa, Aeromonas enteropelogenes
NAAEPIYPDQLRLFSLGEDVCGTDYRPINREEAQSVRNNIVAMMGQWQISGLANNWVILGPGYNGEIKPGKASTTWCYPTRPATAEIPVLPAFNIPDGDAVDVQWRMVHDSANFIKPVSYLAHYLGYAWVGGDHSQFVGDDMDVIQEGDDWVLRGNDGGKCDGYRCNEKSSIRVSNFAYTLDPGSFSHGDVTQSERTLVHTVVGWATNISDTPQSGYDVTLNYTTMSNWSKTNTYGLSEKVSTKNKFKWPLVGETEVSIEIAANQSWASQNGGAVTTALSQSVRPVVPARSRVPVKIELYKANISYPYEFKADMSYDLTFNGFLRWGGNAWHTHPEDRPTLSHTFAIGPFKDKASSIRYQWDKRYLPGEMKWWDWNWAIQQNGLATMQDSLARVLRPVRASITGDFRAESQFAGNIEIGTPVPL

SEQ ID NO: 14 - protein, 420 aa, Aeromonas salmonicida
WHEPVYPDQVKWAGLGTGVCASGYRPLTRDEAMSIKGNLVSRMGQWQITGLADRWVIMGPGYNGEIKQGTAGETWCYPNSPVSGEIPTLSDWNIPAGDEVDVQWRLVHDNDYFIKPVSYLAHYLGYAWVGGNHSPYVGEDMDVTRVGDGWLIKGNNDGGCSGYRCGEKSSIKVSNFSYTLEPDSFSHGQVTESGKQLVKTITANATNYTDLPQQVVVTLKYDKATNWSKTDTYSLSEKVTTKNKFQWPLVGETELAIEIAASQSWASQKGGSTTETVSVEARPTVPPHSSLPVRVALYKSNISYPYEFKAEVNYDLTMKGFLRWGGNAWYTHPDNRPTWEHTFRLGPFRGQGEQHPLPVDKRYIPGEVKWWDWNWTISEYGLSTMQNNLGRVLRPIRSAVTGDFYAESQFAGDIEIGQPQ

SEQ ID NO: 15 - protein, 422 aa, Aeromonas hydrophila
AEPVYPDQLRLFSLGQEVCGDKYRPVNREEAQSIKSNIVGMMGQWQISGLANGWVIMGPGYNGEIKPGSASSTWCYPTNPATGEIPTLSALDIPDGDEVDVQWRLVHDSANFIKPTSYLAHYLGYAWVGGNHSQYVGEDMDVTRDGDGWVIRGNNDGGCDGYRCGDKTSIKVSNFAYNLDPDSFKHGDVTQSDRQLVKTVVGWAINDSDTPQSGYDVTLRYDTATNWSKTNTYGLSEKVTTKNKFKWPLVGETELSIEIAANQSWASQNGGSTTTSLSQSVRPTVPAHSKIPVKIELYKADISYPYEFKADVSYDLTLSGFLRWGGNAWYTHPDNRPNWNHTFVIGPYKDKASSIRYQWDKRYIPGEVKWWDWNWTIQQNGLPTMQNNLAKVLRPVRAGITGDFSAESQFAGNIEIGAPVPV

SEQ ID NO: 16 - protein, 470 aa, synthetic construct
AEPVYPDQLRLFSLGQGVCGDKYRPVNREEAQSVKSNIVGMMGQWQISGLANGWVIMGPGYNGEIKPGTASNTWCYPTNPVTGEIPTLSALDIPDGDEVDVQWRLVHDSANFIKPTSYLAHYLGYAWVGGNHSQYVGEDMDVTRDGDGWVIRGNNDGGCDGYRCGDKTAIKVSNFAYNLDPDSFKHGDVTQSDRQLVKTVVGWAVNDSDTPQSGYDVTLRYDTATNWSKTNTYGLSEAVTTKNKFKWPLVGETELSIEIAANQSWASQNGGSTTTSLSQSVRPTVPARSKIPVKIELYKADISYPYEFKADVSYDLTLSGFLRWGGNAWYTHPDNRPNWNHTFVIGPYKDKASSIRYQWDKRYIPGEVKWWDWNWTIQQNGLSTMQNNLARVLRPVRAGITGDFSAESQFAGNIEIGAPVPLAADSKVRRARSVDGAGQGLRLEIPLDAQELSGLGFNNVSLSVTPAANQ

SEQ ID NO: 17 - protein, 470 aa, synthetic construct
AEPVYPDQLRLFSLGQGVCGDKYRPVNREEAQSVKSNIVGMMGQWQISGLANGWVIMGPGYNGEIKPGTASNTWCYPTNPVTGEIPTLSALDIPDGDEVDVQWRLVHDSANFIKPTSYLAHYLGYAWVGGNHSQYVGEDMDVTRDGDGWVIRGNNDGGCDGYRCGDKTAIKVSNFAYNLDPDSFKHGDVTQSDRQLVKTVVGWAVNDSDTPQSGYDVTLRYDTATNWSKTNTYGLSEAVTTANKFKWPLVGETELSIEIAANQSWASQNGGSTTTSLSQSVRPTVPARSKIPVKIELYKADISYPYEFKADVSYDLTLSGFLRWGGNAWYTHPDNRPNWNHTFVIGPYKDKASSIRYQWDKRYIPGEVKWWDWNWTIQQNGLSTMQNNLARVLRPVRAGITGDFSAESQFAGNIEIGAPVPLAADSKVRRARSVDGAGQGLRLEIPLDAQELSGLGFNNVSLSVTPAANQ

SEQ ID NO: 18 - DNA, 1392 bp, synthetic construct
  source 1..1392: mol_type = other DNA
gcagagcccgtctatccagaccagcttcgcttgttttcattgggccaaggggtctgtggcgacaagtatcgccccgtcaatcgagaagaagcccaaagcgttaaaagcaatattgtcggcatgatggggcaatggcaaataagcgggctggccaacggctgggtcattatggggccgggttataacggtgaaataaaaccagggacagcgtccaatacctggtgttatccgaccaatcctgttaccggtgaaataccgacactgtctgccctggatattccagatggtgacgaagtcgatgtgcagtggcgactggtacatgacagtgcgaatttcatcaaaccaaccagctatctggcccattacctcggttatgcctgggtgggcggcaatcacagccaatatgtcggcgaagacatggatgtgacccgtgatggcgacggctgggtgatccgtggcaacaatgacggcggctgtgacggctatcgctgtggtgacaagacggccatcaaggtcagcaacttcgcctataacctggatcccgacagcttcaagcatggcgatgtcacccagtccgaccgccagctggtcaagactgtggtgggctgggcggtcaacgacagcgacaccccccaatccggctatgacgtcaccctgcgctacgacacagccaccaactggtccaagaccaacacctatggcctgagcgaggccgtgaccaccaagaacaagttcaagtggccactggtgggggaaacccaactctccatcgagattcgtgccaatcagtcctgggcgtcccagaacgggggctcgaccaccacctccctgtctcagtccgtgcgaccgactgtgccggcccgctccaagatcccggtgaagatagagctctacaaggccgacatctcctatccctatgagttcaaggccgatgtcagctatgacctgaccctgagcggcttcctgcgctggggcggcaacgcctggtatacccacccggacaaccgtccgaactggaaccacaccttcgtcataggtccgtacaaggacaaggcgagcagcattcgctaccagtgggacaagcgttacatcccgggtgaagtgaagtggtgggactggaactggaccatacagcagaacggtctgtctaccatgcagaacaacctggccagagtgctgcgcccggtgcgggcggggatcaccggtgatttcagtgccgagagccagtttgccggcaacatagagatcggtgctcccgtgccgctcgcggctgacagcaaggtgcgtcgtgctcgcagtgtggacggcgctggtcaaggcctgaggctggagatcccgctcgatcgcgaagagctctccgggcttggcttcaacaagtcagcctcagcgtga

SEQ ID NO: 19 - DNA, 1392 bp, synthetic construct
  source 1..1392: mol_type = other DNA
gcagagcccgtctatccagaccagcttcgcttgttttcattgggccaaggggtctgtggcgacaagtatcgccccgtcaatcgagaagaagcccaaagcgttaaaagcaatattgtcggcatgatggggcaatggcaaataagcgggctggccaacggctgggtcattatggggccgggttataacggtgaaataaaaccagggacagcgtccaatacctggtgttatccgaccaatcctgttaccggtgaaataccgacactgtctgccctggatattccagatggtgacgaagtcgatgtgcagtggcgactggtacatgacagtgcgaatttcatcaaaccaaccagctatctggcccattacctcggttatgcctgggtgggcggcaatcacagccaatatgtcggcgaagacatggatgtgacccgtgatggcgacggctgggtgatccgtggcaacaatgacggcggctgtgacggctatcgctgtggtgacaagacggccatcaaggtcagcaacttcgcctataacctggatcccgacagcttcaagcatggcgatgtcacccagtccgaccgccagctggtcaagactgtggtgggctgggcggtcaacgacagcgacaccccccaatccggctatgacgtcaccctgcgctacgacacagccaccaactggtccaagaccaacacctatggcctgagcgaggccgtgaccaccgccaacaagttcaagtggccactggtgggggaaacccaactctccatcgagattcgtgccaatcagtcctgggcgtcccagaacgggggctcgaccaccacctccctgtctcagtccgtgcgaccgactgtgccggcccgctccaagatcccggtgaagatagagctctacaaggccgacatctcctatccctatgagttcaaggccgatgtcagctatgacctgaccctgagcggcttcctgcgctggggcggcaacgcctggtatacccacccggacaaccgtccgaactggaaccacaccttcgtcataggtccgtacaaggacaaggcgagcagcattcgctaccagtgggacaagcgttacatcccgggtgaagtgaagtggtgggactggaactggaccatacagcagaacggtctgtctaccatgcagaacaacctggccagagtgctgcgcccggtgcgggcggggatcaccggtgatttcagtgccgagagccagtttgccggcaacatagagatcggtgctcccgtgccgctcgcggctgacagcaaggtgcgtcgtgctcgcagtgtggacggcgctggtcaaggcctgaggctggagatcccgctcgatcgcgaagagctctccgggcttggcttcaacaagtcagcctcagcgtga